European Patent Application EP 4 772 646 A1, published July 8, 2026. Title: 植物培育方法、应用及产物. Applicant: 超级植物（北京）科技有限公司. Application CN. The sequence listing filed with the application follows.

SEQUENCE LISTING (15 sequences)

SEQ ID NO: 1 - protein, 505 aa, Homo sapiens
MKRTPTAEEREREAKKLRLLEELEDTWLPYLTPKDDEFYQQWQLKYPKLILREASSVSEELHKEVQEAFLTLHKHGCLFRDLVRIQGKDLLTPVSRILIGNPGCTYKYLNTRLFTVPWPVKGSNIKHTEAEIAAACETFLKLNDYLQIETIQALEELAAKEKANEDAVPLCMSADFPRVGMGSSYNGQDEVDIKSRAAYNVTLLNFMDPQKMPYLKEEPYFGMGKMAVSWHHDENLVDRSAVAVYSYSCEGPEEESEDDSHLEGRDPDIWHVGFKISWDIETPGLAIPLHQGDCYFMLDDLNATHQHCVLAGSQPRFSSTHRVAECSTGTLDYILQRCQLALQNVCDDVDNDDVSLKSFEPAVLKQGEEIHNEVEFEWLRQFWFQGNRYRKCTDWWCQPMAQLEALWKKMEGVTNAVLHEVKREGLPVEQRNEILTAILASLTARQNLRREWHARCQSRIARTLPADQKPECRPYWEKDDASMPLPFDLTDIVSELRGQLLEAKP

SEQ ID NO: 2 - protein, 505 aa, Sus scrofa
MKRTPTAEERERGAKKLRLLEELEDTWLPYLTPKDDEFYQQWQLKYPKLILREAGSVPEGLHKEVQEAFLALHKHGCLFRDLVRIQGKDLLTPVSRLLIGNPGCTYKYLNTRLFTVPWPVKGSDAKYNEAEIGAACQTFLKLNDYLQIETIQALEELAAKEKANIDTVPACIGPDFPRVGMGSSFDGHDEVDRKSRAAYNLTLLSFMDPQKMPYLKEEPYFGMGKMAVSWHHDENLVDRSAVAVYNYSCEGPEEESEDDPQLEGRNPDVWHVGFKISWDIETPGLAIPLHQGDCYFMLDDLNATHQHCVLAGLPPRFSSTHRVAECSTGALDYILQRCQLALQNVRDEADSGEVSLKSLEPAVLKQGEEIHNEVEFEWLRQFWFQGNRYKKCTDWWCQPMTQLEELWKKMEGATHAVLREVRREGAPVEQSSDILTAILAVLTTRQNLRREWHARCQSRIARTLPVDQKPECRPYWEKDDPSMPLPFDLTDTVAELRGLLLEAKP

SEQ ID NO: 3 - protein, 505 aa, Bos taurus
MKRTPTAEEREREAKKLRLLEELEDTWLPYLTPKDDEFYQQWQLKYPKLILREAASVPELLHKEVQQAFLTLHKHGCLFRDLVRIQGKDLLTPVSRILIGNPGCTYKYLNTRLFTVPWPVKGSDAKYNEAEIAAACQTFLKLNSYLQVETIQALEELAAKEKANIDAVPVCIGPDFPRVGMGSSFDGHDEIDMKNRAAYNVTLLNFMDPQKMPYLKEEPYFGMGKMAVSWHHDENLVDRSAVAVYSYSCEGPEEESEDDPQLEGRDPDIWHVGFKISWDIETPGLAIPLHQGDCYFMLDDLNATHQHCVLAGLPPRFSSTHRVAECSTGTLEYILQRCQVALQNVREEADNGEISLKSLESVVLKQGEEIHNEVEFEWLRQFWFQGSRYKKCTDWWCQPMSQLEEMWRKMEWLTSAVLREVRREGVPMEQKNEMLTSILASITTRQNLRREWHARCQSRIARTLPADQKPECRPYWEKGDPSMPLPFDLTEIVSELRGLLLETRP

SEQ ID NO: 4 - protein, 419 aa, Ostreococcus lucimarinus
MSPSSSVLEPEDGEPFARVHRAHYRGFVVDAPSVLPASLHDDVERAFDDMRSRGEFTHDVVSAGNKVSTTYVRRCLLGEDGMTYHYQKLRLFAQPWRGREAYEVVRRLNETLTRSARERCEKLGGAFAESECEYNVTLINYMETEGESEIELRNEEKFDLGTTSVSWHSDSSLRENSTVAVYHTYEAPERKDWRVALRALNAECEVLCVPLEDKATYYMCGEFNATHHHAVLTGSSARYSSTHRVAVVAKDTFQYIKRRCIDALAIVPDLERENKPLDAKQIQFLADVHREVEFQWIRMFHLQGEAHAAWHDTYWTRKIAELTEAWDRMEACFRVILSKLKRSSRSPESPPRAYAMLLYALKTVKELRDEYTKRTKASAYASLPPSQRPVDLPAYDNTSPLPFELKPVIYFLEEEQNKV

SEQ ID NO: 5 - protein, 522 aa, Aphanomyces astaci
MDPKERKKLERQKKKAKALERKSAKKPNVASLKPVSQPTTSHKRPSEPSGSSAAPPAKKQQIEKAKPLPVPSNYTGPEKFLTPSHPDFHDILTRSYVGFVHEPAAAQPREFHAGMRAAFEHLRDKGYFQYDVVMAGGKHLSRTFVRRTLVGNFGITYKYLGLRIFAHAWDVPSSAAVFRNLYALNQAIVARTKASASPAPPSCEYNLTLINYMEPDNPVLGLKDDLTYDMGKVSVSWHADSSLEDFSSIGVYHTLLPTKKSKKGPCDWRIAMRLSPDVPGAKTTPPLVVPTGDGDVYYLNGDFNHHHQHMVLSGTAVRVSSTHRVAVTAEDTLQYIQAKVTAALKSSAKDPQDKCRRGHADDVRHEQTTVTTLEMDWLRQYWIQGDKHNDLHVDWQQPMLALEASWRKLEARTKTLADALVQSHDVDDLKVLKAVLEGLRNRQVGRDQFVHRMKDKVFKRIAADFQPMERPVWTDWDDVHLLPKDLTATIAALHAHKLVLESEKKRQWKIHAGTRHNKINKA

SEQ ID NO: 6 - protein, 520 aa, Micromonas commode
MGKKHKPRPDDRARVVDASDVGGKVKKKKANGATMKASRRKGGGASANGDGRPYDPSRTLSKPAPPPPAYTPRVPTGAYITPEHDEYDACVARSYVGFVVDPPDILPDELHADVAAAFKTMAKRGLFTRDVLAAGKTVSPTFVSRTLVGERGMTYHYQKLRIFALPWSDEDTPEGSPLRVVRRLNDAMKRRSRALLTRHRDARVPGDVTGSCEFNVTLINLMEPERKESVALKDEGQFGMGKASVSWHSDSSLQDTSTVAVYHQTSGGIDGDDTSWHVALKCLDGVTPALRVPLRSHSAYYIMRDFNLHHHHAVLNGDTRRFSSTHRVAVTAKDTFDYVRGRCERALAVLPSLKWRAGRWPKGTKPPRDASSTQLSDAVRVLGETHREVEFQWIRMFWLQGTRHAAQHDGYWTRRIEELTQAWDVMELGLRFAMDACARAADGKAKAEPRAFEMLRYLLETIAELREEHDARTQSGAYAQVPDDCKPVDLPGFDDSSPLPRNLRPVLNTLERHRRRALDR

SEQ ID NO: 7 - protein, 541 aa, Micromonas pusilla
MATATGSSGGKLEKRKKKKKKTTAVERAGSGGGGNAKKPTTTTASHRPTKPLLRAAPPPPSYRLRGTSGSDDDDDDAAPSFLTPSHAEYERCMKTSYLGFHVDDPSALPEKTHREIARAFERMASDGIFHRDVLAAGKSVSPTFVSRTLLGERGMTYHYQRLRIFAHPWDEETQPDASHPFRAVKRLNDALVSRSTAVLRASSDPRLGDGVDGSCDFNVTLINLMEPASRCAEVPLKDEALFGMGKARSTSVSWHSDSSLQDVSTVAVYHQTDDDDDDSWAVALKTLDGVTPAMRTPLRSREMYYMLRDFNAHHHHAVITGESRRFSSTHRVAVVAKDTFEHIKTRCERALRLLPGIKKIAQVGPGPGDDLAAFARSAQMMGETHRECEFQWIRMFWLQGSRHAASHSAYWRQRIAELTQAWDAMELGYRWALDALRAGASTGAMPLRAYDVVSYLLEETRELRAEHARRSRAGAYEAMPADCRPVDEPKFDEKSPLPFDLGPVLATLAGWRRDAERAQTTTTEGGSKTKKGKPGKGSKRR

SEQ ID NO: 8 - protein, 506 aa, Polarella glacialis
MDMDRFVREPADASSESFHEEFRRCLHGLYEQGIFQYDLIQPVGPGTPVVSTRVTRCLIGEPGITYKYLGLRMFAHPWKGEKTSESCSAMYQHNQELISKAEEQAVAVGCDAPPYSSCFNLTLINRMDPADSGAPNKLGAVSVSWHADSSLVDYSTITVYVAEHDATQDSFGLSPARPCKPCDDPWRVALRHTPNVQGPEKSCPWEVAAQETAKPVKRRAKAKVHTVPIHDGDIYHLIGDFNHHNQHAVLAGRDAVLAVRRGMPVLGGSGTIRYSSTHRVALTEGHSYRSVKQRCSTALSVALADMIPAAAQVHEEQQCSLELEFEWIRQFFIQGKAHREALPWWHSKMDELVFLWRQFEVLTAQRLTLLRRAAAGKVGTSELDPFCLALKNGLQKRAELREAWRQREHDPLLKKQPANRQPLQCLFDAPSDAPHGAGSEALPHNVWPLVEEISQIQLQLHETKKVGKPWYQFVLNVYQGCAFQGGEVTCLSWTLFSQRLPMKRRW

SEQ ID NO: 9 - protein, 543 aa, Guillardia theta
MQETLWQRVKEGLEWFDGAIGEGEEEEEAGRIAGNKGGGRRRGFEQALERYYPKFRVIHRDLLPSALEPSTRRALEVLKDQMGWFRRDYVWVKGKVTQTMVTRLLVGERGCTYKYKGLRLFCRSWETEAAKVPDSACHALAEIRRLNEVLKEKSRKQHECFMARGEGSGEGAVEGGVNSFNATLINYFDESIANHVETRPEPYYGMGRCCISWHADDGVVEQSAIAVYNVIERAEKGEEEELGEVWKVGLKVKWEVDTPGVAVPMVNGDAYVMLSGFNEKNQHCVVCGRGSRFSSTHRVCPQEDMYHNFYCRCRETFLQLHFPWNARGVLQEGEERRACLSKIVASLDALEDLHDQLEFEWLRQFHFQYFDLPPSELDDYWVEVIHVLADLWQRMEIVVWIWISCCRRKSFMVGGKELRDRLERLRQLTSQQKGQGQEVQSSLPFLMKKLLRSEGAGGGREAAGEKAIPEDALELVKATLARRLQKRQEHRIWWEENFRKRLSMGRGGEQREGGKRKRKEGRADGLGFSLLPANLNSLVSTLK

SEQ ID NO: 10 - protein, 420 aa, Ostreococcus tauri
MPDVLGPGDGDAYERVRSFHYDGFVVDDPEILPEALHDDVARAFDSLLREGEFTHDVLSAGNKVSRTFVTRTLLGDRGTTYHYQKLRLFAQPWDGEKRWEYATARRLNEALTRRTREILRGTRHGESECEYNVTLINRMDTREESEVALKDEALFDLGTTSVSWHSDSSLRENSTVAVYSTVDDPERADWSVALRALGKQCPALRVPLKDKATYYMCGDFNATHHHAVLTGSSARYSSTHRVGVVEKDTFQYIKRRCLEALALIPDLENKSASLDAKKIQLLAEIHREVEFQWIRMFHLQGDTHARQHKTYWTQRIAELTEAWDRMEACFRAILSKLKLSPESTPQPSRAYSMMLYAMKEVKELRDEHVKRISASAYAALPESQRPVDLPQYDDTSPLPFELKPVIYFVEAEQAKLKGES

SEQ ID NO: 11 - protein, 787 aa, Ectocarpus sp
MTMTTATTVATTSRLLSPPTSEATTPIQHSNSGMEVSTEKTSHKKKRKSKRKRQQQERDTSSIPDASRQSRGSSSSSTRPPPPPPPPPPTTTTTTTSKKHSRIKEKPARFVHPHLDAELRRLGRSWLSPGDPLFKPALDRSYRGVRHEPGGSLPQAVHRGFRQSFDSLHEAGLFLYDTVQAGGKRLSRTFVTRTLVGDAGITYKYLGLRLFAHPWGLGESDFRKGPGDSLADALNDPCLADLFSNDGSGFDDNDRVADTLRKVGDLSEWMRLRAGAMLKEEVGEAGGERGSCAFNLTLINRMECSGAKRDLKPDPLFSMGKFSVSWHADSCLQDFSTIGVYHCTDPVPAEPDWGIALRVSTEARVGGGGGGSGDGDGYGVSNVEKTRRKEAERGVKPAGPKAIASVAASAAGAVPEKQGEQVLTPPLLIPLQSGDAYFLLDDFNHFHEHAVVSGSSTLRYSSTHRVADTDGNTFSHVQKRCERALAGGGSAAAGGDYHILNLAQVRAEQALLTELESEWLNQFWVQGRRHASLHPWWRGPMALVLATWRELERRTALTVRRLMSLRGQGGGEGVGPGGGGTAAETAGAEPAAIAKAFETVLRALEVRRESRSRWGARFADSAYRSLAADLAPVVPALWPAEGSSGGDVGEEGSPLLLPQSLGGIVSRLRECYTVVYRAASGGKKAGSAKAIAAGAASNWELFRAASSSSSSGGGGAGKKHGSALGKQQQQQQQQQQQQRKMRGLAGQDGLEKTKKRAGGVVKGGGDGGGGRTLKGQGSRRKDRVRER

SEQ ID NO: 12 - protein, 715 aa, Conferva siliculosa
MTTTSATTAARSRLPSPPTSAATTPIQHSNNGTEASPEKTSNKKKAKNKRKRQQECSIPAASQQSRGSSSSSTRPPPPTTTTLKKHSRIKEKPARFVHPHLDAELRRLGRSWLSPGDPLFTPALDRSYRGVRHEPAGSLPQAVHSGFRQSFDSLHEAGLFLYDTVQAGGKRLSRTFVTRTLVGDAGITYKYLGLRLFAHPWGLGESDFRKGPGDGLADALNDPCLADLFSKDGASSVRKSKDNLRGSRFDDNDRVADTLRKVGDLSEWMRLRAGAMLKEEVREAGGERGSCAFNLTLINRMECSGAKRDLKPDPLFSMGKCSVSWHADSCLQDFSTIGVYHCTDPVPAEPDWGIALRVSTEARVGGDGGGDGDGNGVSNDEKTRRKEAERGLKPAGPKAVASVAASAAEAVPEKQGEQVLTPPLLIPLQSGDAYFLLDDFNHFHEHAVVSGSSTLRYSSTHRVADTDGNTFSHVQKRCEQALAGGGSAAAGGDDQILNLAQVRAEQALLTELESEWLNQFWVQGRRHASLHPWWRGPMALVLATWRELERRTSLTVQHLMSLRGQDGGEALWPAEGSGGGDVGEEGSTLLLPQSLGGVISRLRECYTVVYRAASGGKKAGSAKAIAAGAASNWELFRAASSSASSGGGGAGKKHGSALGKQQQQQQQRKKRGAAGQDGLEKKKRAGGVVKGGGDGGGGRTSKGQRSRRKGRVRER

SEQ ID NO: 13 - protein, 417 aa, Fragilariopsis cylindrus
MLTPEDGVYFQKHLQDHYKGFVHLPVDRLEPRDFHEEFKNSLERLRDAGYYQYDVVMAGGKYSSRTFVKRTLVGNPGITYKYLGLRLFAHAWSGPGCTPLMKSIGDMNQSMIKMTEQFPENERCDYNLTLINYMEPTTHTKVGFKDEANYGMGKVSVSWHADSSLVDNSSIGVYHCLPTQRNSKWDWKIALRPLAIESKDNTGSTKRDNKSTTPKPVVVNTKDGDAYFLLGNFNMKHQHCVLAGSQANRISSTHRVAVTIEDTYDYILKRVKIARKRFRLQMETIPPSLQSPVVGLDAKVIRYCQRILTEVEMEWIAQYWLQGDQHDKMRVWWQKPMKTLEAYWCALEVYTYRLFEFLLSRIASNDTVPIDVVKVLIIEFKTRQSFREQWDERRSDKIYQRRVSEEFRPVARPIFEN

SEQ ID NO: 14 - protein, 528 aa, Acanthaster planci
MRFLSLNVLRRWMSKMSKRRQTEDLGKEVKKKKLLSEVARGRLQFLMPDHPDFKSLMRKSYFNFAHEPSTGIPVSLHEELTWALDILRYHGYFYRDWVKVKGQTVQTPISRTLIGEPGTTYKYLGLRLFTIPWSFGHHKPESEVELASETIGKLNEHYKAVSRRLLRKKTAEQTHLKSSPSQEVAPCSSKDRPRERICVEEPKQMTHGLSIEEGTNFNVVLINYMDPEDPDLRLKPEPYYGMGPLAVSWHMDGNLVRGSTVAVYNHTCSSDGGDSTTDSDWMVGFKVSWDIETPGVAIPLQTGESYFMLGDLNDTHQHCVVAGSQARFSTTHRVADCQQGTLSYIQQRCLEALGNLSQLENGEYELKSFQAGHLDFTETVHNEVEFEWLRQFWMQGSRHAAERGGWVPAMECLEADWNKMEHMTKLAVEEANRLGPEEGSVIAEALLPHLKERRKLRQECLDKFPRRLLETIHRDFLPIHRPKWDNDDPSQPLPFDLKGIIRKMRLLCNGKRIKSPSDSESSDTGLHS

SEQ ID NO: 15 - protein, 485 aa, Saccoglossus kowalevskii
MNPRMKRKIPRIPLVTSEGEVAGQLALPIRKQKLLSAVKETQVKFLSPVDTDYKALVAENYDNFVVQPGTELSSELHTRLQQGFETLLTNGYLYQHRIRFRNKTVMTPVSRTLIGEPGMTYRYLNLRLFALPWTFDDKKKLSDVEKACNAFYELNTYFKDHVNKLITEKFASSTGRKIDETDDSLKTIIQRNTEFKATILNYMDPSEIRLKQEPYYNMGDIAVSWHKDESLVDGSTVAVYNHVPMEARQDCSKWKVGLKVAWDITTPAVCTPLNNKDCYYMLDTMNDTHQHCVIAGTLPRYSSTHRVVESSDSTLCYIQQRCQTALDNIGYKDQIPYLKSLETDVLQLIEEIHSEIEFEWLRQFWMQGTQHSQERQYWLKPMEQLQEDWKTMELMTKLMIDIVVKKKDQSHMIAKILLPSLVERNELRNEWMNRYSEKEFYHIPEEHRPIYEPCWTDANSEMPLPFDLSQHIDIIQECMDTNDSQ